European Patent Application EP 4 368 196 A1, published May 15, 2024. Title: AN ANIMAL MODEL OF DISEASES ASSOCIATED WITH LACK OR REDUCTION OF SOCIAL DOMINANCE AND A PHARMACEUTICAL COMPOSITION FOR PREVENTING OR TREATING SAID DISEASES. Applicant: 주식회사 아델. The sequence listing filed with the application follows.

SEQUENCE LISTING (25 sequences)

SEQ ID NO: 1 - DNA, 1860 bp, Mus musculus
  source 1..1860: mol_type = other DNA; note = Mouse CRTC3 DNA
atggccgcctcgcccggttcgggcagcgccaacccgcggaagttcagtgagaagatcgccctgcacacgcagcggcaggccgaggagacgcgggccttcgagcagctcatgaccgacctcaccctgtcccgggttcagtttcagaagcttcagcagctgcgccttacccagtaccacgggggatccttacccaacgtgagccagctgcggaacagcgcgccagagttccagccatcacttcatcaagccgataatgttcgtggaacccgccaccatgggctggtggagaggccagcccggaaccgcttccacccccttcaccgaaggtctggggacaagccagggagacagtttgatgggaatgctttcgcagccagttattcttcacagcacctggatgagagctggccacggcaacagcctccttggaaagaagagaagcatcctggattcaggctaacatctgcacttaacaggaccaattctgattctgctcttcacacgagtgctctgagcaccaaaccccaggacccctatggaggaggaggccagtcagcctggcctgccccatacatgggtttctgtgatggtgaaaacgatggccatgcggaagtagccgccttcccgggtccgctgaaagaagagaatctgttaaatgtcccgaagccactgcctaaacacctgtgggagagcaaggagatccagtccctgtctgggcgccctcgatcctgtgatgttgggggcggcaatgctttcccacataatggccagaacacaggcctctcaccgttcctgggcaccctgaacaccggagggtcgttaccagatctaaccaacctccactactcagcacccctgccagcctccctggacaccagcgaccacctctttggtagcatgagtgtggggaacagcgtgggcaaccttccagctgccatgactcacctggggataagaacctcctctggtctccaaagttctcgaagtaacccttccatccaagccacactcagtaagatggcactctcctcgtccctcaagtgccacccgcagccgtctgtggccaacgcctctgctctgcacccctccctccggctcttctcccttagcaacccgtctctttccaccacaaacctgagtggcccctctcggcgcaggcagcctccagtcagccctctcacgctctctcctggccctgaagcacatcaaggcttcagcagacagctctctgcgaccagcccactgaacccgtatcctgcctcccagatggtgacctcagagcagagcccactttccttcctgcccacagacgctcaagcccaagtgtccccaccacccccttaccccacaccccaggagctgcctcagccactcctacagcagccccatgcccaggagcccccaactcagcagccccaggcagccccctccctgccacagtcagacttccagctcctcactgcccagggctcagctttgaccagcttcttcccggatgtgcgctttgaccaacagcccatgaggcccagccctgcctttcctcagcaggtgcctttggtacagcagagccaccgagaaccacaggactcattccacttgagaccaaacccatattccagctgtggcagcttcccaggcaccatcctgacagaagatacaaacagcaacctgttcaaaggccttagcggggggctgtcgggcatgccagaggtcagcctggacatggacaccccgttccctctggaagaggagctgcagatcgaacccttgagcctcgatggactcaacatgctaagtgactccagcatgggcctgctggacccctctgtggaggagacgtttcgagctgaccggctatga

SEQ ID NO: 2 - protein, 619 aa, Mus musculus
  source 1..619: note = Mouse CRTC3 Protein
MAASPGSGSANPRKFSEKIALHTQRQAEETRAFEQLMTDLTLSRVQFQKLQQLRLTQYHGGSLPNVSQLRNSAPEFQPSLHQADNVRGTRHHGLVERPARNRFHPLHRRSGDKPGRQFDGNAFAASYSSQHLDESWPRQQPPWKEEKHPGFRLTSALNRTNSDSALHTSALSTKPQDPYGGGGQSAWPAPYMGFCDGENDGHAEVAAFPGPLKEENLLNVPKPLPKHLWESKEIQSLSGRPRSCDVGGGNAFPHNGQNTGLSPFLGTLNTGGSLPDLTNLHYSAPLPASLDTSDHLFGSMSVGNSVGNLPAAMTHLGIRTSSGLQSSRSNPSIQATLSKMALSSSLKCHPQPSVANASALHPSLRLFSLSNPSLSTTNLSGPSRRRQPPVSPLTLSPGPEAHQGFSRQLSATSPLNPYPASQMVTSEQSPLSFLPTDAQAQVSPPPPYPTPQELPQPLLQQPHAQEPPTQQPQAAPSLPQSDFQLLTAQGSALTSFFPDVRFDQQPMRPSPAFPQQVPLVQQSHREPQDSFHLRPNPYSSCGSFPGTILTEDTNSNLFKGLSGGLSGMPEVSLDMDTPFPLEEELQIEPLSLDGLNMLSDSSMGLLDPSVEETFRADRL

SEQ ID NO: 3 - DNA, 1857 bp, Rattus norvegicus
  source 1..1857: mol_type = other DNA; note = Rat CRTC3 DNA
atggccgcctcgcccggctcgggcagcgccaacccgcggaagttcagtgagaagatcgcgctgcacacgcagcggcaggccgaggagacgcgggccttcgagcagctcatgaccgacctcaccctgtcccgggttcagtttcagaggcttcagcaactgcgccttacacagcaccacgggggatccttacctaatgtgagccagctgcggggcagcgcaccagagcttcagccgtcactccatcacgctgataatgtccgtgggacccgccaccatgggctggtggagaggccagcccggaaccgcttccaccctcttcaccgcaggtctggggacaagccagggagacagtttgatggaaatgcttttgcagccagttattcttcgcagcccctggatgagagctggccaaggcaacagcctccatggaaagaggaaaagcatcctggattcaggctgacatctgcacttaacaggaccaattctgattctgctcttcacacgagtgctctgagcaccaaaccccaggacccctatggaggaggaggccagtcagcctggcctgccccatacatgggtttctgtgatggtgaaaatgatggccgtggggaagccgccttccccggtctgctgaaggaagagaatctgttaaacgtcccgaagccactgcccaaacaactgtgggagaccaaggagatccagtccctgtctggacgccctcggtcctgtgatgttgggggcggcagtgccttcccacataatggccaaaacacaggcctctcgccatttctggggaccctgaacactggagggtcattaccagatctaaccaaccttcactactcagcacccctgccagcctccctggacaccagtgaccacctctttggtagcatgagcgtggggaacagtgtgggcaaccttccagctgctatgactcacctggggataagaaactcctctggtctccagagttctcgaagtaacccttccatccaagccacgctcaataagattgcgctgtcctcatccctcaatagccacccacagccgtccgtggccaatgcctctgctctccacccctcgctccgtctcttctcccttagcaacccatctctttctaccacaaacctgagtggcccctctcggcgcaggcagcctccagtcagccctctcacgctctctcctggccctgaagcacatcaaggtttcaacagacagctatctgcaaccagcccactgaacccgtaccctgcctcccagatggtgacctcagagcagagtccactttccttcctgcccacagacgctcaagcccaagtgtccccaccacccccttaccccacaccccaggagctgcctcaaccactcctacagcagccccatgcccatgagcccccagctcagcagccccaggcagccccctccctgtcacagtcagacttccagctcctcactgcccagggctcgtctctgaccaacttcttccgcgatgtgggctttgaccagcagcccatgaggcccagccccgcctttcctcagcaggtgcctttggtacagcagagccaccgagaaccacaggactcgttccacttgagaccaaacccatattccaactgtgggagcttcccgaacaccatcctgacagaagataccaacaccagcctgttcaaaggccttagtggggggctgtcgggcatgcctgaggtcagcctggacatggacactccgttcccgctggaagaggagctacagatcgaacccttgagcctggacggactcaacatgttaagtgactccagcatgggcctgctggacccctctgtggaggagacatttcgagctgaccggctgtga

SEQ ID NO: 4 - protein, 618 aa, Rattus norvegicus
  source 1..618: note = Rat CRTC3 Protein
MAASPGSGSANPRKFSEKIALHTQRQAEETRAFEQLMTDLTLSRVQFQRLQQLRLTQHHGGSLPNVSQLRGSAPELQPSLHHADNVRGTRHHGLVERPARNRFHPLHRRSGDKPGRQFDGNAFAASYSSQPLDESWPRQQPPWKEEKHPGFRLTSALNRTNSDSALHTSALSTKPQDPYGGGGQSAWPAPYMGFCDGENDGRGEAAFPGLLKEENLLNVPKPLPKQLWETKEIQSLSGRPRSCDVGGGSAFPHNGQNTGLSPFLGTLNTGGSLPDLTNLHYSAPLPASLDTSDHLFGSMSVGNSVGNLPAAMTHLGIRNSSGLQSSRSNPSIQATLNKIALSSSLNSHPQPSVANASALHPSLRLFSLSNPSLSTTNLSGPSRRRQPPVSPLTLSPGPEAHQGFNRQLSATSPLNPYPASQMVTSEQSPLSFLPTDAQAQVSPPPPYPTPQELPQPLLQQPHAHEPPAQQPQAAPSLSQSDFQLLTAQGSSLTNFFRDVGFDQQPMRPSPAFPQQVPLVQQSHREPQDSFHLRPNPYSNCGSFPNTILTEDTNTSLFKGLSGGLSGMPEVSLDMDTPFPLEEELQIEPLSLDGLNMLSDSSMGLLDPSVEETFRADRL

SEQ ID NO: 5 - DNA, 1860 bp, Macaca mulatta
  source 1..1860: mol_type = other DNA; note = Monkey CRTC3 DNA
atggccgcctcgccgggctcgggcagcgccaacccgcggaagttcagtgagaagatcgcgctgcacacgcagcgacaggccgaggagacgcgggccttcgagcagctcatgaccgacctcaccctgtcgcgggttcaatttcagaagcttcagcaactgcgccttacacagtaccatggaggatccttaccaaatgtgagccagctgcggagcagtgcgtcagagtttcagccgtcatttcaccaagctgataatgttcggggaacccgccatcacgggctggtggagaggccatccaggaaccgcttccaccccctgcaccgaaggtctggggacaagccagggcggcaatttgatggtagtgcttttggagccaattattcctcacagcctctggatgagagttggccaaggcagcagcctccttggaaagacgaaaagcatcctgggttcaggctgacatctgcacttaacaggaccaattctgattctgctcttcacacgagtgctctgagcaccaagccccaggacccctatggaggagggggccagtcggcctggcctgccccatacatgggtttctgtgatggtgagaataatggacatggggaagtagcatctttccctggcccattgaaagaagagaatctgttaaatgttccgaagccagtgccaaaacaactgtgggagaccaaggagattcaatccctgtcaggacgccctcgatcctgtgatgttggaggtggcaatgcttttccacataatggtcaaaacctaggcctttcaccctttttggggaccctgaatactggagggtcattgccagatctaaccaacctccactactccacgcccctgccagcctccctgaacaccaccgaccacctcttcgggagtatgagtgtggggaatagtgtgaacaacatcccagctgctgtgacccacctgggtataagaagctcctctggtctccagagttctcggagtaacccctccatccaagccacgctcaataagactgtgctttcctcttccctaaataaccacccgcagacatctgttcccaatgcatctgctcttcacccttcactccgtctattttcccttagcaacccatctctttccaccacaaacctgagtggcccatctcggcgtcggcagcctcccgtcagtcctctcaccctttctcctggccccgaagcacatcaaggtttcagcagacagctgtcttcaaccagcccactggccccatatcctacctcccagatggtgtcctcagaccgaagccaactttccttcctgcccacagaagctcaagcccaggtgtccccgccacccccttaccctgcgccccaggagctcacccagcccctcctgcagcagccccgcacccctgaggcccctgcccagcagccccaggcagcctcctcactgccacagtcggactttcagcttctcccagcccagggctcatctttgaccaacttcttcccagatgtgggttttgaccagcagtccatgaggccaggccctgcctttcctcaacaggtgcctctagtgcaacaaggttcccgagaactgcaggactcttttcatttgagaccaagcccatattccaactgcgggagtttcccaaacaccatcctgacagaagactccagcaccagcctgttcaaagacctcaacagtgcgctcgcaggcctgcccgaggtcagcctgaacgtggacactccatttccactggaagaggagctgcagattgaacccctgagcctggacggactcaacatgttaagtgactccagcatgggcctgctggacccctctgttgaagagacgtttcgagctgacagactgtga

SEQ ID NO: 6 - protein, 619 aa, Macaca mulatta
  source 1..619: note = Monkey CRTC3 Protein
MAASPGSGSANPRKFSEKIALHTQRQAEETRAFEQLMTDLTLSRVQFQKLQQLRLTQYHGGSLPNVSQLRSSASEFQPSFHQADNVRGTRHHGLVERPSRNRFHPLHRRSGDKPGRQFDGSAFGANYSSQPLDESWPRQQPPWKDEKHPGFRLTSALNRTNSDSALHTSALSTKPQDPYGGGGQSAWPAPYMGFCDGENNGHGEVASFPGPLKEENLLNVPKPVPKQLWETKEIQSLSGRPRSCDVGGGNAFPHNGQNLGLSPFLGTLNTGGSLPDLTNLHYSTPLPASLNTTDHLFGSMSVGNSVNNIPAAVTHLGIRSSSGLQSSRSNPSIQATLNKTVLSSSLNNHPQTSVPNASALHPSLRLFSLSNPSLSTTNLSGPSRRRQPPVSPLTLSPGPEAHQGFSRQLSSTSPLAPYPTSQMVSSDRSQLSFLPTEAQAQVSPPPPYPAPQELTQPLLQQPRTPEAPAQQPQAASSLPQSDFQLLPAQGSSLTNFFPDVGFDQQSMRPGPAFPQQVPLVQQGSRELQDSFHLRPSPYSNCGSFPNTILTEDSSTSLFKDLNSALAGLPEVSLNVDTPFPLEEELQIEPLSLDGLNMLSDSSMGLLDPSVEETFRADRL

SEQ ID NO: 7 - DNA, 756 bp, Homo sapiens
  source 1..756: mol_type = other DNA; note = Human AREG DNA
atgagagccccgctgctaccgccggcgccggtggtgctgtcgctcttgatactcggctcaggccattatgctgctggattggacctcaatgacacctactctgggaagcgtgaaccattttctggggaccacagtgctgatggatttgaggttacctcaagaagtgagatgtcttcagggagtgagatttcccctgtgagtgaaatgccttctagtagtgaaccgtcctcgggagccgactatgactactcagaagagtatgataacgaaccacaaatacctggctatattgtcgatgattcagtcagagttgaacaggtagttaagcccccccaaaacaagacggaaagtgaaaatacttcagataaacccaaaagaaagaaaaagggaggcaaaaatggaaaaaatagaagaaacagaaagaagaaaaatccatgtaatgcagaatttcaaaatttctgcattcacggagaatgcaaatatatagagcacctggaagcagtaacatgcaaatgtcagcaagaatatttcggtgaacggtgtggggaaaagtccatgaaaactcacagcatgattgacagtagtttatcaaaaattgcattagcagccatagctgcctttatgtctgctgtgatcctcacagctgttgctgttattacagtccagcttagaagacaatacgtcaggaaatatgaaggagaagctgaggaacgaaagaaacttcgacaagagaatggaaatgtacatgctatagca

SEQ ID NO: 8 - protein, 98 aa, Homo sapiens
  source 1..98: note = Human AREG Protein
SVRVEQVVKPPQNKTESENTSDKPKRKKKGGKNGKNRRNRKKKNPCNAEFQNFCIHGECKYIEHLEAVTCKCQQEYFGERCGEKSMKTHSMIDSSLSK

SEQ ID NO: 9 - DNA, 123 bp, Homo sapiens
  source 1..123: mol_type = other DNA; note = Human AREG-EGF DNA
aagaaaaatccatgtaatgcagaatttcaaaatttctgcattcacggagaatgcaaatatatagagcacctggaagcagtaacatgcaaatgtcagcaagaatatttcggtgaacggtgtggg

SEQ ID NO: 10 - protein, 41 aa, Homo sapiens
  source 1..41: note = Human AREG-EGF Protein
KKNPCNAEFQNFCIHGECKYIEHLEAVTCKCQQEYFGERCG

SEQ ID NO: 11 - protein, 98 aa, Mus musculus
  source 1..98: note = Mouse AREG Protein
SVRVEQVIKPKKNKTEGEKSTEKPKRKKKGGKNGKGRRNKKKKNPCTAKFQNFCIHGECRYIENLEVVTCNCHQDYFGERCGEKSMKTHSEDDKDLSK

SEQ ID NO: 12 - protein, 53 aa, Mus musculus
  source 1..53: note = Mouse EGF Protein
NSYPGCPSSYDGYCLNGGVCMHIESLDSYTCNCVIGYSGDRCQTRDLRWWELR

SEQ ID NO: 13 - protein, 43 aa, synthetic construct
  source 1..43: note = AREG-EGF Peptide
KKNPCNAEFQNFCIHGECKYIEHLEAVTCKCQQEYFGERCGEK

SEQ ID NO: 14 - protein, 41 aa, synthetic construct
  source 1..41: note = AREG-HB Peptide
SVRVEQVVKPPQNKTESENTSDKPKRKKKGGKNGKNRRNRK

SEQ ID NO: 15 - DNA, 20 bp, synthetic construct
  source 1..20: mol_type = other DNA; note = Forward primer for CRTC3 WT mouse
cctgagttattggcggatgt

SEQ ID NO: 16 - DNA, 20 bp, synthetic construct
  source 1..20: mol_type = other DNA; note = Reverse primer for CRTC3 WT mouse
cactcaggctgtagcaagca

SEQ ID NO: 17 - DNA, 20 bp, synthetic construct
  source 1..20: mol_type = other DNA; note = Forward primer for CRTC3 KO mouse
atggaaggattggagctacg

SEQ ID NO: 18 - DNA, 20 bp, synthetic construct
  source 1..20: mol_type = other DNA; note = Reverse primer for CRTC3 KO mouse
cactcaggctgtagcaagca

SEQ ID NO: 19 - DNA, 23 bp, synthetic construct
  source 1..23: mol_type = other DNA; note = Forward primer for mouse GAPDH
ccatcaccatcttccaggagcga

SEQ ID NO: 20 - DNA, 23 bp, synthetic construct
  source 1..23: mol_type = other DNA; note = Reverse primer for mouse GAPDH
ggatgaccttgcccacagccttg

SEQ ID NO: 21 - DNA, 22 bp, synthetic construct
  source 1..22: mol_type = other DNA; note = Forward primer for mouse CRTC3
cttcacagcacctggatgagag

SEQ ID NO: 22 - DNA, 22 bp, synthetic construct
  source 1..22: mol_type = other DNA; note = Reverse primer for mouse CRTC3
tgctcagagcactcgtgtgaag

SEQ ID NO: 23 - DNA, 24 bp, synthetic construct
  source 1..24: mol_type = other DNA; note = Forward primer for mouse AREG
gccattatgcagctgctttggacg

SEQ ID NO: 24 - DNA, 24 bp, synthetic construct
  source 1..24: mol_type = other DNA; note = Reverse primer for mouse AREG
tgtttttcttgggcttaatcacct

SEQ ID NO: 25 - DNA, 402 bp, synthetic construct
  source 1..402: mol_type = other DNA; note = mAREG 94-191 for AAV5-GFAP-mAREG construct
atgagaactccgctgctaccgctggcgcgctcagtgctgttgctgctggtcttaggctcaggccattatgcagctgcttcagtcagagttgaacaggtgattaagcccaagaaaaacaagacagaaggagaaaagtctacagaaaaacccaaaaggaagaaaaagggaggcaaaaatggaaaaggcagaaggaataagaagaaaaagaatccatgcactgccaagtttcagaacttttgcattcatggcgaatgcagatacatcgagaacctggaggtggtgacatgcaattgtcatcaagattactttggtgaacggtgtggagaaaaatccatgaagactcacagcgaggatgacaaggacctatccaagtacccatacgatgttccagattacgcttag